European Patent Application EP 4 520 835 A1, published March 12, 2025. Title: A process for preparing a composition comprising apocarotenoids and compositions obtained thereby. Applicant: Universitaet Stuttgart. Application EP. The sequence listing filed with the application follows.

SEQUENCE LISTING (9 sequences)

SEQ ID NO: 1 - protein, 498 aa, Capsicum annuum
MDTLLRTPNNLEFLHGFGVKVSAFSSVKSQKFGAKKFCEGLGSRSVCVKASSSALLELVPETKKENLDFELPMYDPSKGVVVDLAVVGGGPAGLAVAQQVSEAGLSVCSIDPNPKLIWPNNYGVWVDEFEAMDLLDCLDATWSGATVYIDDNTTKDLNRPYGRVNRKQLKSKMMQKCILNGVKFHQAKVIKVIHEESKSMLICNDGITIQATVVLDATGFSRSLVQYDKPYNPGYQVAYGILAEVEEHPFDVNKMVFMDWRDSHLKNNVELKERNSRIPTFLYAMPFSSNRIFLEETSLVARPGLGMDDIQERMVARLSHLGIKVKSIEEDEHCVIPMGGPLPVLPQRVVGIGGTAGMVHPSTGYMVARTLAAAPVVANAIIQYLSSERSHSGDELSAAVWKDLWPIERRRQREFFCFGMDILLKLDLPATRRFFDAFFDLEPRYWHGFLSSRLFLPELIVFGLSLFSHASNTSRLEIMTKGTLPLVHMINNLLQDKE

SEQ ID NO: 2 - protein, 369 aa, Arabidopsis thaliana
MDLLDCLDTTWSGAVVYVDEGVKKDLSRPYGRVNRKQLKSKMLQKCITNGVKFHQSKVTNVVHEEANSTVVCSDGVKIQASVVLDATGFSRCLVQYDKPYNPGYQVAYGIVAEVDGHPFDVDKMVFMDWRDKHLDSYPELKERNSKIPTFLYAMPFSSNRIFLEETSLVARPGLRMEDIQERMAARLKHLGINVKRIEEDERCVIPMGGPLPVLPQRVVGIGGTAGMVHPSTGYMVARTLAAAPIVANAIVRYLGSPSSNSLRGDQLSAEVWRDLWPIERRRQREFFCFGMDILLKLDLDATRRFFDAFFDLQPHYWHGFLSSRLFLPELLVFGLSLFSHASNTSRLEIMTKGTVPLAKMINNLVQDRD

SEQ ID NO: 3 - protein, 524 aa, Arabidopsis thaliana
MECVGARNFAAMAVSTFPSWSCRRKFPVVKRYSYRNIRFGLCSVRASGGGSSGSESCVAVREDFADEEDFVKAGGSEILFVQMQQNKDMDEQSKLVDKLPPISIGDGALDLVVIGCGPAGLALAAESAKLGLKVGLIGPDLPFTNNYGVWEDEFNDLGLQKCIEHVWRETIVYLDDDKPITIGRAYGRVSRRLLHEELLRRCVESGVSYLSSKVDSITEASDGLRLVACDDNNVIPCRLATVASGAASGKLLQYEVGGPRVCVQTAYGVEVEVENSPYDPDQMVFMDYRDYTNEKVRSLEAEYPTFLYAMPMTKSRLFFEETCLASKDVMPFDLLKTKLMLRLDTLGIRILKTYEEEWSYIPVGGSLPNTEQKNLAFGAAASMVHPATGYSVVRSLSEAPKYASVIAEILREETTKQINSNISRQAWDTLWPPERKRQRAFFLFGLALIVQFDTEGIRSFFRTFFRLPKWMWQGFLGSTLTSGDLVLFALYMFVISPNNLRKGLINHLISDPTGATMIKTYLKV

SEQ ID NO: 4 - protein, 537 aa, Zea mays
MGLSGATISAPLGCCVLRCGAVGGGKALKADAERWRRAGWSRRVGGPKVRCVATEKHDETAAVGAAVGVDFADEEDYRKGGGGELLYVQMQSTKPMESQSKIASKLSPISDENTVLDLVIIGCGPAGLSLASESAKKGLTVGLIGPDLPFTNNYGVWEDEFKDLGLESCIEHVWKDTIVYLDNNKPILIGRSYGRVHRDLLHEELLKRCYEAGVTYLNSKVDKIIESPDGHRVVCCDKGREIICRLAIVASGAASGRLLEYEVGGPRVCVQTAYGVEVEVENNPYDPSLMVFMDYRDCFKEEFSHTEQENPTFLYAMPMSPTRVFFEETCLASKDAMSFDLLKKRLMYRLNAMGIRILKVYEEEWSYIPVGGSLPNTDQKNLAFGAAASMVHPATGYSVVRSLSEAPRYASVISDILGNRVPAEYMLGNSQNYSPSMLAWRTLWPQERKRQRSFFLFGLALIIQLNNEGIQTFFEAFFRVPRWMWRGFLGSTLSSVDLILFSFYMFAIAPNQLRMNLVRHLLSDPTGSSMIKTYLTL

SEQ ID NO: 5 - protein, 552 aa, Dunaliella salina strain
MNSLQISSGSHLASAPRHSLKNSCNARWTRDKGGRQGPPRALKTKVEAPPQTQNTRSREHEDVNQLIREGHYEKPSVQAQASKRDSAQQSLASTLTPATPSSLYDVAVVGAGPAGMYLAAELSNRGLRTVIIGHDSPLVNNYGVWIDEARSLGLEHTLDNAWDDAVCYFKEGHKVNLGRGYGRVSRRKLREHLLRLCTDAGVEFLKGEVANMELTSDGKQTCLDVKNGPQMHARLVTLAAGAAAGKFLRYEEDAPGVAAQTAYGIEAEVENYDQVYPAGEMLFMDFRRHHTGVWDGAASRIKSGAHPAGDNNLWGTRGEVPSFRYAMPLGGNRVFLEETCLVAKPALPFKVLKRRLERRLKAMGVRVKEVHEEEWSYIPVGGPLPEGNQPITAFGAAANLVHPATGFSVSRSFREAPGLADQIAASLRKPDQSVQQTAAQVWEALWPQEKRTQTSFHVFGMELLASLDLADTNLFFETFFKLPKSMWQGYMASKLSSLQLISFAFLTFVLASPRIKMLLVASLLSDPAGAYVFNAYKKLYIKSQEEKELSEP

SEQ ID NO: 6 - protein, 382 aa, Pantoea ananas
MQPHYDLILVGAGLANGLIALRLQQQQPDMRILLIDAAPQAGGNHTWSFHHDDLTESQHRWIAPLVVHHWPDYQVRFPTRRRKLNSGYFCITSQRFAEVLQRQFGPHLWMDTAVAEVNAESVRLKKGQVIGARAVIDGRGYAANSALSVGFQAFIGQEWRLSHPHGLSSPIIMDATVDQQNGYRFVYSLPLSPTRLLIEDTHYIDNATLDPECARQNICDYAAQQGWQLQTLLREEQGALPITLSGNADAFWQQRPLACSGLRAGLFHPTTGYSLPLAVAVADRLSALDVFTSASIHHAITHFARERWQQQGFFRMLNRMLFLAGPADSRWRVMQRFYGLPEDLIARFYAGKLTLTDRLRILSGKPPVPVLAALQAIMTTHR

SEQ ID NO: 7 - protein, 411 aa, Synechococcus elongatus
MFDALVIGSGPAGLAIAAELAQRGLKVQGLSPVDPFHPWENTYGIWGPELDSLGLEHLFGHRWSNCVSYFGEAPVQHQYNYGLFDRAQLQQHWLRQCEQGGLQWQLGKAAAIAHDSHHSCVTTAAGQELQARLVVDTTGHQAAFIQRPHSDAIAYQAAYGIIGQFSQPPIEPHQFVLMDYRSDHLSPEERQLPPTFLYAMDLGNDVYFVEETSLAACPAIPYDRLKQRLYQRLATRGVTVQVIQHEEYCLFPMNLPLPDLTQSVVGFGGAASMVHPASGYMVGALLRRAPDLANAIAAGLNASSSLTTAELATQAWRGLWPTEKIRKHYIYQFGLEKLMRFSEAQLNHHFQTFFGLPKEQWYGFLTNTLSLPELIQAMLRLFAQAPNDVRWGLMEQQGRELQLFWQAIAAR

SEQ ID NO: 8 - protein, 532 aa, Camellia sinensis var. assamica
MECIGARNFAAMAVSTCPIWRYRKKRQRNTLTRVIHRHSSYTSSLRVRSSSAGSESCVAFEEGFADEEDYIKAGGSELLFVQMQQNKLMEKQSKLADKLPPISVGNTILDLVVIGCGPAGLALAAESAKLGLSVGLIGPDLPFTNNYGVWEDEFRDLGLEGCIEHVWGDTIVYLDDNDSPFLIGPCFIGRVSRYLLHEELVKRCVESGVSYLSSKVERIIESAIGHSLIECEQNVVVPCRLATVASGAASGKLLQYEVGGPRVSVQTAYGMEVEVENNPYDPNLMVFMDYRDYVKPRVQCLEAQYPTFLYAMPMSPTRVFFEETCLASKDAMPFDLLKKKLMSRLETMGVRVIKTYEEEWSYIPVGGSLPNTEQKNLALGAAASMVHPATGYFVVRSLSEAPKYASVIANILKQGHSRDKLSRSWSTENISMLAWNTLWPQERKRQRAFFLFGLALILQLDIDGIRTFFHTFFRLPTWMWQGFLGSTLSSADLALFAFYMFVIAPNNMRMCLVRHLLSDPTGATMIRTYLTI

SEQ ID NO: 9 - protein, 500 aa, Solanum lycopersicum
MDTLLKTPNNLEFLNPHHGFAVKASTFRSEKHHNFGSRKFCETLGRSVCVKGSSSALLELVPETKKENLDFELPMYDPSKGVVVDLAVVGGGPAGLAVAQQVSEAGLSVCSIDPNPKLIWPNNYGVWVDEFEAMDLLDCLDATWSGAAVYIDDNTAKDLHRPYGRVNRKQLKSKMMQKCIMNGVKFHQAKVIKVIHEESKSMLICNDGITIQATVVLDATGFSRSLVQYDKPYNPGYQVAYGILAEVEEHPFDVNKMVFMDWRDSHLKNNTDLKERNSRIPTFLYAMPFSSNRIFLEETSLVARPGLRIDDIQERMVARLNHLGIKVKSIEEDEHCLIPMGGPLPVLPQRVVGIGGTAGMVHPSTGYMVARTLAAAPVVANAIIQYLGSERSHSGNELSTAVWKDLWPIERRRQREFFCFGMDILLKLDLPATRRFFDAFFDLEPRYWHGFLSSRLFLPELIVFGLSLFSHASNTSRFEIMTKGTVPLVNMINNLLQDKE